European Patent Application EP 4 393 939 A1, published July 3, 2024. Title: LYSE VARIANT AND METHOD FOR PRODUCING L-ARGININE BY USING SAME. Applicant: CJ CheilJedang Corporation. The sequence listing filed with the application follows.

SEQUENCE LISTING (40 sequences)

SEQ ID NO: 1 - protein, 233 aa, Corynebacterium sp.
MEIFITGLLLGASLLLSIGPQNVLVIKQGIKREGLIAVLLVCLISDVFLFIAGTLGVDLLSNAAPIVLDIMRWGGIAYLLWFAVMAAKDAMTNKVEAPQIIEETEPTVPDDTPLGGSAVATDTRNRVRVEVSVDKQRVWVKPMLMAIVLTWLNPNAYLDAFVFIGGVGAQYGDTGRWIFAAGAFAASLIWFPLVGFGAAALSRPLSSPKVWRWINVVVAVVMTALAIKLMLMG

SEQ ID NO: 2 - DNA, 702 bp, Corynebacterium sp.
  source 1..702: mol_type = genomic DNA
atggaaatcttcattacaggtctgcttttgggggccagtcttttgctgtccatcggaccgcagaatgtactggtgattaaacaaggaattaagcgcgaaggactcattgcggttcttctcgtgtgtttaatttctgacgtctttttgttcatcgccggcaccttgggcgttgatcttttgtccaatgccgcgccgatcgtgctcgatattatgcgctggggtggcatcgcttacctgttatggtttgccgtcatggcagcgaaagacgccatgacaaacaaggtggaagcgccacagatcattgaagaaacagaaccaaccgtgcccgatgacacgcctttgggcggttcggcggtggccactgacacgcgcaaccgggtgcgggtggaggtgagcgtcgataagcagcgggtttgggtgaagcccatgttgatggcaatcgtgctgacctggttgaacccgaatgcgtatttggacgcgtttgtgtttatcggcggcgtcggcgcgcaatacggcgacaccggacggtggattttcgccgctggcgcgttcgcggcaagcctgatctggttcccgctggtgggtttcggcgcagcagcattgtcacgcccgctgtccagccccaaggtgtggcgctggatcaacgtcgtcgtggcagttgtgatgaccgcattggccatcaaactgatgttgatgggttag

SEQ ID NO: 3 - DNA, 34 bp, synthetic construct
  misc_feature 1..34: note = primer_lysE-AF
  source 1..34: mol_type = other DNA
tcggtacccggggatcccgcttcatcttccaagc

SEQ ID NO: 4 - DNA, 34 bp, synthetic construct
  misc_feature 1..34: note = primer_lysE-BR
  source 1..34: mol_type = other DNA
tgcaggtcgactctagagagaacttgttgcagtc

SEQ ID NO: 5 - DNA, 35 bp, synthetic construct
  misc_feature 1..35: note = primer_lysE-F50L-AR
  source 1..35: mol_type = other DNA
aaggtgccggcgatgagcaaaaagacgtcagaaat

SEQ ID NO: 6 - DNA, 35 bp, synthetic construct
  misc_feature 1..35: note = primer_lysE-F50L-BF
  source 1..35: mol_type = other DNA
ctcatcgccggcaccttgggcgttgatcttttgtc

SEQ ID NO: 7 - DNA, 35 bp, synthetic construct
  misc_feature 1..35: note = primer_lysE-F50I-AR
  source 1..35: mol_type = other DNA
aaggtgccggcgatgatcaaaaagacgtcagaaat

SEQ ID NO: 8 - DNA, 35 bp, synthetic construct
  misc_feature 1..35: note = primer_lysE-F50I-BF
  source 1..35: mol_type = other DNA
atcatcgccggcaccttgggcgttgatcttttgtc

SEQ ID NO: 9 - DNA, 35 bp, synthetic construct
  misc_feature 1..35: note = primer_lysE-F50V-AR
  source 1..35: mol_type = other DNA
aaggtgccggcgatgaccaaaaagacgtcagaaat

SEQ ID NO: 10 - DNA, 35 bp, synthetic construct
  misc_feature 1..35: note = primer_lysE-F50V-BF
  source 1..35: mol_type = other DNA
gtcatcgccggcaccttgggcgttgatcttttgtc

SEQ ID NO: 11 - DNA, 35 bp, synthetic construct
  misc_feature 1..35: note = primer_lysE-N153S-AR
  source 1..35: mol_type = other DNA
cattcgggctcaaccaggtcagcacgattgccatc

SEQ ID NO: 12 - DNA, 35 bp, synthetic construct
  misc_feature 1..35: note = primer_lysE-N153S-BF
  source 1..35: mol_type = other DNA
ctggttgagcccgaatgcgtatttggacgcgtttg

SEQ ID NO: 13 - DNA, 35 bp, synthetic construct
  misc_feature 1..35: note = primer_lysE-N153T-AR
  source 1..35: mol_type = other DNA
cattcggggtcaaccaggtcagcacgattgccatc

SEQ ID NO: 14 - DNA, 35 bp, synthetic construct
  misc_feature 1..35: note = primer_lysE-N153T-BF
  source 1..35: mol_type = other DNA
ctggttgaccccgaatgcgtatttggacgcgtttg

SEQ ID NO: 15 - DNA, 35 bp, synthetic construct
  misc_feature 1..35: note = primer_lysE-N153Q-AR
  source 1..35: mol_type = other DNA
cattcggttgcaaccaggtcagcacgattgccatc

SEQ ID NO: 16 - DNA, 35 bp, synthetic construct
  misc_feature 1..35: note = primer_lysE-N153Q-BF
  source 1..35: mol_type = other DNA
ctggttgcaaccgaatgcgtatttggacgcgtttg

SEQ ID NO: 17 - DNA, 35 bp, synthetic construct
  misc_feature 1..35: note = primer_lysE-N215T-AR
  source 1..35: mol_type = other DNA
cgacgacggtgatccagcgccacaccttggggctg

SEQ ID NO: 18 - DNA, 34 bp, synthetic construct
  misc_feature 1..34: note = primer_lysE-N215T-BF
  source 1..34: mol_type = other DNA
ctggatcaccgtcgtcgtggcagttgtgatgacc

SEQ ID NO: 19 - DNA, 35 bp, synthetic construct
  misc_feature 1..35: note = primer_lysE-N215S-AR
  source 1..35: mol_type = other DNA
cgacgacgctgatccagcgccacaccttggggctg

SEQ ID NO: 20 - DNA, 34 bp, synthetic construct
  misc_feature 1..34: note = primer_lysE-N215S-BF
  source 1..34: mol_type = other DNA
ctggatcagcgtcgtcgtggcagttgtgatgacc

SEQ ID NO: 21 - DNA, 35 bp, synthetic construct
  misc_feature 1..35: note = primer_lysE-N215Q-AR
  source 1..35: mol_type = other DNA
cgacgacttggatccagcgccacaccttggggctg

SEQ ID NO: 22 - DNA, 34 bp, synthetic construct
  misc_feature 1..34: note = primer_lysE-N215Q-BF
  source 1..34: mol_type = other DNA
ctggatccaagtcgtcgtggcagttgtgatgacc

SEQ ID NO: 23 - DNA, 36 bp, synthetic construct
  misc_feature 1..36: note = primer_argR-AF
  source 1..36: mol_type = other DNA
tcggtacccggggatccagcaggccttaagggtaag

SEQ ID NO: 24 - DNA, 34 bp, synthetic construct
  misc_feature 1..34: note = primer_argR-AR
  source 1..34: mol_type = other DNA
aggggcgctgtcttacctcggctggtgggccagc

SEQ ID NO: 25 - DNA, 36 bp, synthetic construct
  misc_feature 1..36: note = primer_argR-BF
  source 1..36: mol_type = other DNA
ggtaagacagcgcccctagttcaaggcttgttaatc

SEQ ID NO: 26 - DNA, 37 bp, synthetic construct
  misc_feature 1..37: note = primer_argR-BR
  source 1..37: mol_type = other DNA
tgcaggtcgactctagaaccgttgaactgcttgccag

SEQ ID NO: 27 - protein, 233 aa, synthetic construct
  REGION 1..233: note = LysE F50L
MEIFITGLLLGASLLLSIGPQNVLVIKQGIKREGLIAVLLVCLISDVFLLIAGTLGVDLLSNAAPIVLDIMRWGGIAYLLWFAVMAAKDAMTNKVEAPQIIEETEPTVPDDTPLGGSAVATDTRNRVRVEVSVDKQRVWVKPMLMAIVLTWLNPNAYLDAFVFIGGVGAQYGDTGRWIFAAGAFAASLIWFPLVGFGAAALSRPLSSPKVWRWINVVVAVVMTALAIKLMLMG

SEQ ID NO: 28 - protein, 233 aa, synthetic construct
  REGION 1..233: note = LysE N153S
MEIFITGLLLGASLLLSIGPQNVLVIKQGIKREGLIAVLLVCLISDVFLFIAGTLGVDLLSNAAPIVLDIMRWGGIAYLLWFAVMAAKDAMTNKVEAPQIIEETEPTVPDDTPLGGSAVATDTRNRVRVEVSVDKQRVWVKPMLMAIVLTWLSPNAYLDAFVFIGGVGAQYGDTGRWIFAAGAFAASLIWFPLVGFGAAALSRPLSSPKVWRWINVVVAVVMTALAIKLMLMG

SEQ ID NO: 29 - protein, 233 aa, synthetic construct
  REGION 1..233: note = LysE N215T
MEIFITGLLLGASLLLSIGPQNVLVIKQGIKREGLIAVLLVCLISDVFLFIAGTLGVDLLSNAAPIVLDIMRWGGIAYLLWFAVMAAKDAMTNKVEAPQIIEETEPTVPDDTPLGGSAVATDTRNRVRVEVSVDKQRVWVKPMLMAIVLTWLNPNAYLDAFVFIGGVGAQYGDTGRWIFAAGAFAASLIWFPLVGFGAAALSRPLSSPKVWRWITVVVAVVMTALAIKLMLMG

SEQ ID NO: 30 - protein, 233 aa, synthetic construct
  REGION 1..233: note = LysE F50I
MEIFITGLLLGASLLLSIGPQNVLVIKQGIKREGLIAVLLVCLISDVFLIIAGTLGVDLLSNAAPIVLDIMRWGGIAYLLWFAVMAAKDAMTNKVEAPQIIEETEPTVPDDTPLGGSAVATDTRNRVRVEVSVDKQRVWVKPMLMAIVLTWLNPNAYLDAFVFIGGVGAQYGDTGRWIFAAGAFAASLIWFPLVGFGAAALSRPLSSPKVWRWINVVVAVVMTALAIKLMLMG

SEQ ID NO: 31 - protein, 233 aa, synthetic construct
  REGION 1..233: note = LysE F50V
MEIFITGLLLGASLLLSIGPQNVLVIKQGIKREGLIAVLLVCLISDVFLVIAGTLGVDLLSNAAPIVLDIMRWGGIAYLLWFAVMAAKDAMTNKVEAPQIIEETEPTVPDDTPLGGSAVATDTRNRVRVEVSVDKQRVWVKPMLMAIVLTWLNPNAYLDAFVFIGGVGAQYGDTGRWIFAAGAFAASLIWFPLVGFGAAALSRPLSSPKVWRWINVVVAVVMTALAIKLMLMG

SEQ ID NO: 32 - protein, 233 aa, synthetic construct
  REGION 1..233: note = LysE N153T
MEIFITGLLLGASLLLSIGPQNVLVIKQGIKREGLIAVLLVCLISDVFLFIAGTLGVDLLSNAAPIVLDIMRWGGIAYLLWFAVMAAKDAMTNKVEAPQIIEETEPTVPDDTPLGGSAVATDTRNRVRVEVSVDKQRVWVKPMLMAIVLTWLTPNAYLDAFVFIGGVGAQYGDTGRWIFAAGAFAASLIWFPLVGFGAAALSRPLSSPKVWRWINVVVAVVMTALAIKLMLMG

SEQ ID NO: 33 - protein, 233 aa, synthetic construct
  REGION 1..233: note = LysE N153Q
MEIFITGLLLGASLLLSIGPQNVLVIKQGIKREGLIAVLLVCLISDVFLFIAGTLGVDLLSNAAPIVLDIMRWGGIAYLLWFAVMAAKDAMTNKVEAPQIIEETEPTVPDDTPLGGSAVATDTRNRVRVEVSVDKQRVWVKPMLMAIVLTWLQPNAYLDAFVFIGGVGAQYGDTGRWIFAAGAFAASLIWFPLVGFGAAALSRPLSSPKVWRWINVVVAVVMTALAIKLMLMG

SEQ ID NO: 34 - protein, 233 aa, synthetic construct
  REGION 1..233: note = LysE N215S
MEIFITGLLLGASLLLSIGPQNVLVIKQGIKREGLIAVLLVCLISDVFLFIAGTLGVDLLSNAAPIVLDIMRWGGIAYLLWFAVMAAKDAMTNKVEAPQIIEETEPTVPDDTPLGGSAVATDTRNRVRVEVSVDKQRVWVKPMLMAIVLTWLNPNAYLDAFVFIGGVGAQYGDTGRWIFAAGAFAASLIWFPLVGFGAAALSRPLSSPKVWRWISVVVAVVMTALAIKLMLMG

SEQ ID NO: 35 - protein, 233 aa, synthetic construct
  REGION 1..233: note = LysE N215Q
MEIFITGLLLGASLLLSIGPQNVLVIKQGIKREGLIAVLLVCLISDVFLFIAGTLGVDLLSNAAPIVLDIMRWGGIAYLLWFAVMAAKDAMTNKVEAPQIIEETEPTVPDDTPLGGSAVATDTRNRVRVEVSVDKQRVWVKPMLMAIVLTWLNPNAYLDAFVFIGGVGAQYGDTGRWIFAAGAFAASLIWFPLVGFGAAALSRPLSSPKVWRWIQVVVAVVMTALAIKLMLMG

SEQ ID NO: 36 - DNA, 702 bp, synthetic construct
  misc_feature 1..702: note = LysE F50L nt
  source 1..702: mol_type = other DNA
atggaaatcttcattacaggtctgcttttgggggccagtcttttgctgtccatcggaccgcagaatgtactggtgattaaacaaggaattaagcgcgaaggactcattgcggttcttctcgtgtgtttaatttctgacgtctttttgctcatcgccggcaccttgggcgttgatcttttgtccaatgccgcgccgatcgtgctcgatattatgcgctggggtggcatcgcttacctgttatggtttgccgtcatggcagcgaaagacgccatgacaaacaaggtggaagcgccacagatcattgaagaaacagaaccaaccgtgcccgatgacacgcctttgggcggttcggcggtggccactgacacgcgcaaccgggtgcgggtggaggtgagcgtcgataagcagcgggtttgggtgaagcccatgttgatggcaatcgtgctgacctggttgaacccgaatgcgtatttggacgcgtttgtgtttatcggcggcgtcggcgcgcaatacggcgacaccggacggtggattttcgccgctggcgcgttcgcggcaagcctgatctggttcccgctggtgggtttcggcgcagcagcattgtcacgcccgctgtccagccccaaggtgtggcgctggatcaacgtcgtcgtggcagttgtgatgaccgcattggccatcaaactgatgttgatgggttag

SEQ ID NO: 37 - DNA, 702 bp, synthetic construct
  misc_feature 1..702: note = LysE N153S nt
  source 1..702: mol_type = other DNA
atggaaatcttcattacaggtctgcttttgggggccagtcttttgctgtccatcggaccgcagaatgtactggtgattaaacaaggaattaagcgcgaaggactcattgcggttcttctcgtgtgtttaatttctgacgtctttttgttcatcgccggcaccttgggcgttgatcttttgtccaatgccgcgccgatcgtgctcgatattatgcgctggggtggcatcgcttacctgttatggtttgccgtcatggcagcgaaagacgccatgacaaacaaggtggaagcgccacagatcattgaagaaacagaaccaaccgtgcccgatgacacgcctttgggcggttcggcggtggccactgacacgcgcaaccgggtgcgggtggaggtgagcgtcgataagcagcgggtttgggtgaagcccatgttgatggcaatcgtgctgacctggttgagcccgaatgcgtatttggacgcgtttgtgtttatcggcggcgtcggcgcgcaatacggcgacaccggacggtggattttcgccgctggcgcgttcgcggcaagcctgatctggttcccgctggtgggtttcggcgcagcagcattgtcacgcccgctgtccagccccaaggtgtggcgctggatcaacgtcgtcgtggcagttgtgatgaccgcattggccatcaaactgatgttgatgggttag

SEQ ID NO: 38 - DNA, 702 bp, synthetic construct
  misc_feature 1..702: note = LysE N215T nt
  source 1..702: mol_type = other DNA
atggaaatcttcattacaggtctgcttttgggggccagtcttttgctgtccatcggaccgcagaatgtactggtgattaaacaaggaattaagcgcgaaggactcattgcggttcttctcgtgtgtttaatttctgacgtctttttgttcatcgccggcaccttgggcgttgatcttttgtccaatgccgcgccgatcgtgctcgatattatgcgctggggtggcatcgcttacctgttatggtttgccgtcatggcagcgaaagacgccatgacaaacaaggtggaagcgccacagatcattgaagaaacagaaccaaccgtgcccgatgacacgcctttgggcggttcggcggtggccactgacacgcgcaaccgggtgcgggtggaggtgagcgtcgataagcagcgggtttgggtgaagcccatgttgatggcaatcgtgctgacctggttgaacccgaatgcgtatttggacgcgtttgtgtttatcggcggcgtcggcgcgcaatacggcgacaccggacggtggattttcgccgctggcgcgttcgcggcaagcctgatctggttcccgctggtgggtttcggcgcagcagcattgtcacgcccgctgtccagccccaaggtgtggcgctggatcaccgtcgtcgtggcagttgtgatgaccgcattggccatcaaactgatgttgatgggttag

SEQ ID NO: 39 - protein, 171 aa, Corynebacterium sp.
MSLGSTPSTPENLNPVTRTARQALILQILDKQKVTSQVQLSELLLDEGIDITQATLSRDLDELGARKVRPDGGRAYYAVGPVDSIAREDLRGPSEKLRRMLDELLVSTDHSGNIAMLRTPPGAAQYLASFIDRVGLKEVVGTIAGDDTVFVLARDPLTGKELGELLSGRTT

SEQ ID NO: 40 - DNA, 516 bp, Corynebacterium sp.
  source 1..516: mol_type = genomic DNA
atgtcccttggctcaaccccgtcaacaccggaaaacttaaatcccgtgactcgcactgcacgccaagctctcattttgcagattttggacaaacaaaaagtcaccagccaggtacaactgtctgaattgctgctggatgaaggcatcgatatcacccaggccaccttgtcccgagatctcgatgaactcggtgcacgcaaggttcgccccgatgggggacgcgcctactacgcggtcggcccagtagatagcatcgcccgcgaagatctccggggtccgtcggagaagctgcgccgcatgcttgatgaactgctggtttctacagatcattccggcaacatcgcgatgctgcgcaccccgccgggagctgcccagtacctggcaagtttcatcgatagggtggggctgaaagaagtcgttggcaccatcgctggcgatgacaccgttttcgttctcgcccgtgatccgctcacaggtaaagaactaggtgaattactcagcgggcgcaccacttaa